European Patent Application EP 4 265 636 A1, published October 25, 2023. Title: Preparation of target peptides and proteins. Applicant: mk2 Biotechnologies GmbH. The sequence listing filed with the application follows.

SEQUENCE LISTING (13 sequences)

SEQ ID NO: 1 - protein, 9 aa, Artificial Sequence
  Nonapeptide
GGAGNDTLY

SEQ ID NO: 2 - protein, 68 aa, Artificial Sequence
  Capping sequence (CAP)
INAGADQLWFARQGNDLEIRILGTDDALTVHDWYRDADHRVEIIHAANQAVDQAGIEKLVEAMAQYPD

SEQ ID NO: 3 - protein, 168 aa, Classical swine fever virus
MELNHFELLYKTSKQKPVGVEEPVYDTAGRPLFGNPSEVHPQSTLKLPHDRGRGDIRTTLRDLPRKGDCRSGNHLGPVSGIYIKPGPVYYQDYTGPVYHRAPLEFFDEAQFCEVTKRIGRVTGSDGKLYHIYVCVDGCILLKLAKRGTPRTLKWIRNFTNCPLWVTSC

SEQ ID NO: 4 - protein, 168 aa, Artificial Sequence
  CSFV NPro EDDIE
MELNHFELLYKTSKQKPVGVEEPVYDTAGRPLFGNPSEVHPQSTLKLPHDRGEDDIETTLRDLPRKGDCRSGNHLGPVSGIYIKPGPVYYQDYTGPVYHRAPLEFFDETQFEETTKRIGRVTGSDGKLYHIYVEVDGEILLKQAKRGTPRTLKWTRNTTNCPLWVTSC

SEQ ID NO: 5 - protein, 152 aa, Artificial Sequence
  CSFV Delta 1-16 NPro EDDIE derivative
PVGVEEPVYDTAGRPLFGNPSEVHPQSTLKLPHDRGEDDIETTLRDLPRKGDCRSGNHLGPVSGIYIKPGPVYYQDYTGPVYHRAPLEFFDETQFEETTKRIGRVTGSDGKLYHIYVEVDGEILLKQAKRGTPRTLKWTRNTTNCPLWVTSC

SEQ ID NO: 6 - protein, 6 aa, Artificial Sequence
  Nickel-assisted cleavage tag 1
SRHWAP

SEQ ID NO: 7 - protein, 5 aa, Artificial Sequence
  Nickel-assisted cleavage tag 2
GSHHW

SEQ ID NO: 8 - DNA, 744 bp, Artificial Sequence
  Coding sequence for (GGAGNDTLY)7-Delta 1-16 Npro EDDIE-Lfc
atgggcggagcggggaatgatacgctgtatggcggcgcgggcaacgacactttgtacggtggtgccgggaatgacaccctgtatggtggcgcagggaacgacacgctgtatggtggtgcgggaaatgacaccctttatggcggtgcaggcaacgataccttatatggaggcgcgggtaacgacaccctttacccagtcggcgtagaagaaccggtgtatgataccgctggtcgtccactgtttggtaacccgagtgaagtgcatccgcaatccacgctcaaactgccgcatgatcgtggggaagatgatatcgagacaaccttgcgggatttaccgcgcaaaggggattgtcgctcaggcaaccacttaggtcccgttagcgggatctacatcaaaccaggtcctgtctactatcaggactataccggcccggtttatcatcgcgctcccctggagttcttcgatgagacacagtttgaagaaacgacgaaacgcattggccgtgtgactggctctgatggcaaactgtaccacatttacgtcgaagtggatggcgaaattctcctgaaacaggccaaacgcggtacccctcgcactctgaagtggactcgcaataccaccaattgtccgctgtgggttactagttgcttcaagtgccgtcgttggcaatggcgcatgaagaaactgggagcaccgtcgattacatgcgtacggcgtgcctttcaccatcatcaccaccattaa

SEQ ID NO: 9 - protein, 247 aa, Artificial Sequence
  (GGAGNDTLY)7-Delta 1-16 Npro EDDIE-Lfc
MGGAGNDTLYGGAGNDTLYGGAGNDTLYGGAGNDTLYGGAGNDTLYGGAGNDTLYGGAGNDTLYPVGVEEPVYDTAGRPLFGNPSEVHPQSTLKLPHDRGEDDIETTLRDLPRKGDCRSGNHLGPVSGIYIKPGPVYYQDYTGPVYHRAPLEFFDETQFEETTKRIGRVTGSDGKLYHIYVEVDGEILLKQAKRGTPRTLKWTRNTTNCPLWVTSCFKCRRWQWRMKKLGAPSITCVRRAFHHHHHH

SEQ ID NO: 10 - DNA, 918 bp, Artificial Sequence
  Coding sequence for Lfc-SRHWAP-(GGAGNDTLY)17-CAP
atgcatcatcaccatcaccacttcaaatgtcgtcgctggcaatggcggatgaagaaacttggcgcaccgagcattacttgcgttcgtcgcgcattttcccgtcattgggcgcctactagtggtggagcgggtaatgacacgttgtatggtggggccgggaatgatacgttatatggcggcgccggtaatgacaccttatatggtggagccggtaacgacacgctgtatggtggagctggtaatgacacactgtatggtggcgcgggtaacgatacgttgtatggcggggctggcaacgatacgctgtacggcggcgccggcaatgacacactttacggcggggcaggaaatgataccctttacggtggcgcggggaacgataccctgtatggcggagcgggcaatgacactctgtacggtggcgctggcaacgacacattgtatggcggagctggtaacgacaccttatacggtggggcgggcaacgataccttgtatggtggcgctggtaacgatactctctacggcggcgcgggcaatgataccctctatggaggggcaggcaacgatactctgtacatcaatgcaggcgccgaccagctgtggtttgcgcggcaagggaacgatctggaaattcgcattctggggaccgatgatgccctgaccgtgcatgattggtaccgcgatgcggaccatcgcgtcgaaattatccacgcagctaaccaggcagtagatcaggccggtatcgagaaactggtggaagcgatggcgcagtatccggatcaccatcatcaccaccataataacaacgatctgttccaggcgtcacgtcgccgctttctggcccaactgggtggtttaaccgttgccggcatgctgggtccgagtctgctcaccccacgtcgcgcctctgcgtaa

SEQ ID NO: 11 - protein, 305 aa, Artificial Sequence
  Lfc-SRHWAP-(GGAGNDTLY)17-CAP
MHHHHHHFKCRRWQWRMKKLGAPSITCVRRAFSRHWAPTSGGAGNDTLYGGAGNDTLYGGAGNDTLYGGAGNDTLYGGAGNDTLYGGAGNDTLYGGAGNDTLYGGAGNDTLYGGAGNDTLYGGAGNDTLYGGAGNDTLYGGAGNDTLYGGAGNDTLYGGAGNDTLYGGAGNDTLYGGAGNDTLYGGAGNDTLYINAGADQLWFARQGNDLEIRILGTDDALTVHDWYRDADHRVEIIHAANQAVDQAGIEKLVEAMAQYPDHHHHHHNNNDLFQASRRRFLAQLGGLTVAGMLGPSLLTPRRASA

SEQ ID NO: 12 - DNA, 1167 bp, Artificial Sequence
  Coding sequence for FGF2-SRHWAP-(GGAGNDTLY)17-CAP
atgcatcaccatcaccaccatccagccctgcccgaagatggcggatcaggtgcatttccacccggtcacttcaaagatccgaaacgcctctactgcaagaatggaggcttctttctgcggattcatccggatggtcgcgttgatggggtgcgtgaaaagagcgaccctcatatcaaactgcagttgcaggccgaagaacgtggtgtggtcagcatcaaaggcgtttgtgccaaccgctatctggcgatgaaagaggatggtcgcttgctggcgtccaaatgtgtgaccgatgaatgcttcttctttgaacgcctggaatcgaataactacaatacatatcgctctcgcaagtacagttcgtggtatgtcgcgctgaagcgtacgggtcagtataaactggggccgaaaactggacctggccagaaagcgattctgtttctcccgatgtccgcgaaaagcagtcggcattgggcgccgacctctggtggcgcgggaaacgacaccctgtatggcggggctggtaatgataccctgtatggtggggccggcaatgataccttatacggtggtgcagggaacgataccttatatggcggtgcaggcaacgatacgctgtacggaggggcgggaaatgatacgctttatggtggtgccggcaacgacacgttgtatggcggcgctggaaatgacactctttacggtggggcaggcaatgacaccttgtacggcggtgcgggtaatgatactctgtatggcggcgcgggtaacgacacgttatatggtggcgcaggcaacgacacactgtacggcggcgcaggcaatgataccctctatggcggtgcggggaacgataccctgtacggaggtgctggtaacgacactctgtacggtggcgccggcaacgatacattatatggcggggcgggcaatgacaccctttacatcaacgctggtgctgatcagctttggtttgcgcgtcaaggcaacgacctggaaattcgtattctcggcaccgatgacgctctgacggtgcatgattggtatcgtgatgccgaccatcgcgtagagatcattcatgcagcgaaccaagccgtagatcaagccgggattgagaaactggttgaggccatggcacagtatccggatcaccatcatcaccaccactaa

SEQ ID NO: 13 - protein, 388 aa, Artificial Sequence
  FGF2-SRHWAP-(GGAGNDTLY)17-CAP
MHHHHHHPALPEDGGSGAFPPGHFKDPKRLYCKNGGFFLRIHPDGRVDGVREKSDPHIKLQLQAEERGVVSIKGVCANRYLAMKEDGRLLASKCVTDECFFFERLESNNYNTYRSRKYSSWYVALKRTGQYKLGPKTGPGQKAILFLPMSAKSSRHWAPTSGGAGNDTLYGGAGNDTLYGGAGNDTLYGGAGNDTLYGGAGNDTLYGGAGNDTLYGGAGNDTLYGGAGNDTLYGGAGNDTLYGGAGNDTLYGGAGNDTLYGGAGNDTLYGGAGNDTLYGGAGNDTLYGGAGNDTLYGGAGNDTLYGGAGNDTLYINAGADQLWFARQGNDLEIRILGTDDALTVHDWYRDADHRVEIIHAANQAVDQAGIEKLVEAMAQYPDHHHHHH